European Patent Specification EP 3 210 996 B1, published August 9, 2023. Title: Peptides Enhancing Neuronal Outgrowth and Application Thereof. Applicant: SCHWEITZER BIOTECH COMPANY LTD. The sequence listing filed with the application follows.

SEQUENCE LISTING (9 sequences)

SEQ ID NO: 1 - protein, 5 aa, Artificial Sequence
  Peptide for enhancing neuronal outgrowth
NAIPQ

SEQ ID NO: 2 - protein, 5 aa, Artificial Sequence
  Peptide for enhancing neuronal outgrowth
NPSPQ

SEQ ID NO: 3 - protein, 85 aa, Artificial Sequence
  Peptide for enhancing neuronal outgrowth
  MOD_RES (1)..(40): Xaa = any amino acid, Xaa at positions 1-40 may be present or absent
  MOD_RES (42)..(42): Xaa = any nonpolar amino acid
  MOD_RES (43)..(43): Xaa = any amino acid
  MOD_RES (46)..(85): Xaa = any amino acid, Xaa at positions 46-85 may be present or absent
XXXXXXXXXXXXXXXXXXXXXXXXXXXXXXXXXXXXXXXXNXXPQXXXXXXXXXXXXXXXXXXXXXXXXXXXXXXXXXXXXXXXX

SEQ ID NO: 4 - protein, 5 aa, Artificial Sequence
  Petide for enhancing neuronal outgrowth
NFEPQ

SEQ ID NO: 5 - protein, 5 aa, Artificial Sequence
  Petide for enhancing neuronal outgrowth
NMYPQ

SEQ ID NO: 6 - protein, 5 aa, Artificial Sequence
  Petide for enhancing neuronal outgrowth
NIKPQ

SEQ ID NO: 7 - protein, 5 aa, Artificial Sequence
  Petide for enhancing neuronal outgrowth
NLMPQ

SEQ ID NO: 8 - protein, 5 aa, Artificial Sequence
  Petide for enhancing neuronal outgrowth
NVAPQ

SEQ ID NO: 9 - protein, 5 aa, Artificial Sequence
  Petide for enhancing neuronal outgrowth
NWLPQ